European Patent Specification EP 3 559 226 B1, published January 4, 2023. Title: BACILLUS GIBSONII-CLADE SERINE PROTEASES. Applicant: DANISCO US INC. Babe, Lilia Maria Dankmeyer, Lydia Goedegebuur, Frits Kaper, Thijs Mulder, Harm Pricelius, Sina. The sequence listing filed with the application follows.

SEQUENCE LISTING (13 sequences)

SEQ ID NO: 1 - protein, 269 aa, Bacillus gibsonii
QQTVPWGITRVQAPAVHNRGITGSGVRVAILDSGISAHSDLNIRGGASFVPGEPTTADLNGHGTHVAGTVAALNNSIGVIGVAPNAELYAVKVLGANGSGSVSGIAQGLEWAATNNMHIANMSLGSDFPSSTLERAVNYATSRDVLVIAATGNNGSGSVGYPARYANAMAVGATDQNNRRANFSQYGTGIDIVAPGVNVQSTYPGNRYVSMNGTSMATPHVAGAAALVKQRYPSWNATQIRNHLKNTATNLGNSSQFGSGLVNAEAATR

SEQ ID NO: 2 - DNA, 1052 bp, Bacillus subtilis
gcaaaacgcggatcattggaagagacgaccgtacccgcagcatcaatgcctaaaataagcggatactctctgacgatattgcctcctgcttttccggccagaccatctttgtaattaatgccggaataagcaactttaatcaggacaccatccttcggcaaatcctctgttgatatggttttcacatggactgaaacatcatcggcatttttttctgcctgcaaggcttgaaataacgttgacattcggcacactccttttcatttatatcgtaaccgaagaacgttcaaaaaaccaaatcatcaagccgccattttcacttcgccggcacattgagacaataatggacaaatccggtatcctcttcatagccgttttgctcatacaagcttcttgccttccggttgtggtgctcagtctgaagtgttaaacattttgccccgttttgccctgcataatcctttgcggcagaaagcagccggccgccggctccctttgtacgcgcatgaggaacgacaaataagtcatttaatatgtatatccttttcattgacacagaagaaaacgttggatagagctgggtaaagcctatgaattctccattttcttctgctatcaaaataacagactcgtgattttccaaacgagctttcaaaaaagcctctgccccttgcaaatcggatgcctgtctataaaattcccgatattggttaaacagcggcgcaatggcggccgcatctgatgtctttgcttggcgaatgttcatcttatttcttcctccctctcaataattttttcattctatcccttttctgtaaagtttatttttcagaatacttttatcatcatgctttgaaaaaatatcacgataatatccattgttctcacggaagcacacgcgtcgctgataaacagctgacatcaactaaaagcttcattaaatactttgaaaaaagttgttgacttaaaagaagctaaatgttatagtaataaaacagaatagtcttttaagtaagtctactctgaatttttttaaaaggagagggtaaaga

SEQ ID NO: 3 - DNA, 87 bp, Bacillus subtilis
gtgagaagcaaaaaattgtggatcagcttgttgtttgcgttaacgttaatctttacgatggcgttcagcaacatgtctgcgcaggct

SEQ ID NO: 4 - DNA, 252 bp, Bacillus lentus
gctgaagaagcaaaagaaaaatatttaattggctttaatgagcaggaagctgtcagtgagtttgtagaacaagtagaggcaaatgacgaggtcgccattctctctgaggaagaggaagtcgaaattgaattgcttcatgaatttgaaacgattcctgttttatccgttgagttaagcccagaagatgtggacgcgcttgaactcgatccagcgatttcttatattgaagaggatgcagaagtaacgacaatg

SEQ ID NO: 5 - DNA, 810 bp, Artificial Sequence
  variant DNA sequence
caacaaacagtgccatggggaattactcgtgtgcaagccccagctgttcataaccgtggaattacaggttctggtgtaagagttgctatcctcgattcaggtatttccacacatgaagacttaaatgttcgtggtggcgttagctttgtaccaggggaaccaacgtatgctgatttaaatgggcatggcacgcatgtggctgggacggtagctgctttaaacaattcgattggcgttgttggcgtagcaccgtcagcggatctatacgctgttaaagtattaggggcgaatggtagaggttcggtcagcgggattgcccaaggattggaatgggcagcacaaaataacatgcacattgctaatatgagtttaggaacagatgcaccaagttctacacttgagcgtgctgttaattatgcgacttctagagatgttcttgttattgcggcaactgggaataacggttctggctcagtaggctatccggcccgttatgcgaacgcaatggcagtcggagctactgaccaaaacaacagacgcgccaacttttcacagtatggcacggggattgacattgtcgcaccaggtgtaaacgtgcagagcacatacccaggtaaccgttatgtgagcatgaacggtacatcgatggctactcctcatgttgcaggtgcagcagcccttgttaaacaacgctatccatcttggaatgcgactcaaatccgcgaccatctaaagaatacggcaacgaatttaggaaactcttcacaatttggaagcggacttgtcaatgcagaagcggcaacacgctaa

SEQ ID NO: 6 - DNA, 254 bp, Bacillus amyloliquefaciens
tctagatacataaaaaaccggccttggccccgccggttttttattatttttcttcctccgcatgttcaatccgctccataatcgacggatggctccctctgaaaattttaacgagaaacggcgggttgacccggctcagtcccgtaacggccaagtcctgaaacgtctcaatcgccgcttcccggtttccggtcagctcaatgccgtaacggtcggcggcgttttcctgataccgggagacggcattcgtaatc

SEQ ID NO: 7 - DNA, 855 bp, Staphylococcus aureus
ttagtgacattagaaaaccgactgtaaaaagtacagtcggcattatctcatattataaaagccagtcattaggcctatctgacaattcctgaatagagttcataaacaatcctgcatgataaccatcacaaacagaatgatgtacctgtaaagatagcggtaaatatattgaattacctttattaatgaattttcctgctgtaataatgggtagaaggtaattactattattattgatatttaagttaaacccagtaaatgaagtccatggaataatagaaagagaaaaagcattttcaggtataggtgttttgggaaacaatttccccgaaccattatatttctctacatcagaaaggtataaatcataaaactctttgaagtcattctttacaggagtccaaataccagagaatgttttagatacaccatcaaaaattgtataaagtggctctaacttatcccaataacctaactctccgtcgctattgtaaccagttctaaaagctgtatttgagtttatcacccttgtcactaagaaaataaatgcagggtaaaatttatatccttcttgttttatgtttcggtataaaacactaatatcaatttctgtggttatactaaaagtcgtttgttggttcaaataatgattaaatatctcttttctcttccaattgtctaaatcaattttattaaagttcatttgatatgcctcctaaatttttatctaaagtgaatttaggaggcttacttgtctgctttcttcattagaatcaatccttttttaaaagtcaatattactgtaacataaatatatattttaaaaatatcccactttatccaattttcgtttgt

SEQ ID NO: 8 - protein, 269 aa, Artificial Sequence
  variant of Bgi02446
QQTVPWGITRVQAPAVHNRGITGSGVRVAILDSGISTHEDLNVRGGVSFVPGEPTYADLNGHGTHVAGTVAALNNSIGVVGVAPSADLYAVKVLGANGRGSVSGIAQGLEWAAQNNMHIANMSLGTDAPSSTLERAVNYATSRDVLVIAATGNNGSGSVGYPARYANAMAVGATDQNNRRANFSQYGTGIDIVAPGVNVQSTYPGNRYVSMNGTSMATPHVAGAAALVKQRYPSWNATQIRDHLKNTATNLGNSSQFGSGLVNAEAATR

SEQ ID NO: 9 - DNA, 994 bp, Artificial Sequence
  3' flanking region
tcagccttattctcctgataacgcgagacagcattagaaaaaggcgtaaccgcaaagctcaaaacagaaaacaaaagcaataacagcggaagtgccgcaagatcatgccgcccttctaaatgaaacatgctgcgggttaggcgaaccgtccgcttgtaaagcttatcaatgacataaaatccggcgagcgacacgagcaaatagccagccagaccgatgtaaacgtgcttcatgacataatggcccatttcgtggcccataataaacagaatttctgaatcgtcaagtttgttcagcgtcgtatcccacaatacaatccgtttattggccccaattcctgtaacataggcattcagcgcatttgttttttctgacatgttcacttcatatacatggtcagccggaatattggcttcatctgccagctctaaaattttgctttcaagctctttgtttttcagcggataaaaatcattgtataaaggatcgataatgaccggctgaataaaaaacagaaacagcgaaaacggcactgttaacagccaggcgtataaccaccattttttttcatgccttttgatcagccaataaaaaacgagaacgcaaagcgtaaagattggaaagctgatccaaaagctgataacctgatccttagcccagctggccgttgtctgtgtggaaatgttatagtcaagcgatacttgatagcctatccaatctaaaggcagcgtcaccaatgttgtaatcagcgaaagcacaaacacaaaaccaacggtctgcaaaaaccgaaaaggcacggccgcttcgatccatttcttgattttctttgaaacaccgctgacaagcagaacaaaaaacagaaaccaatcaagtggtaccccgataaaaaataaaaaattcttgacattcgaatactgctcggccactgccaactcagacggcttcatgaaagaagccggatcagcctgcgtccctttcacggcttccggtattg

SEQ ID NO: 10 - protein, 29 aa, Bacillus subtilis
VRSKKLWISLLFALTLIFTMAFSNMSAQA

SEQ ID NO: 11 - protein, 84 aa, Bacillus lentus
AEEAKEKYLIGFNEQEAVSEFVEQVEANDEVAILSEEEEVEIELLHEFETIPVLSVELSPEDVDALELDPAISYIEEDAEVTTM

SEQ ID NO: 12 - DNA, 602 bp, Bacillus subtilis
tccattttcttctgctatcaaaataacagactcgtgattttccaaacgagctttcaaaaaagcctctgccccttgcaaatcggatgcctgtctataaaattcccgatattggttaaacagcggcgcaatggcggccgcatctgatgtctttgcttggcgaatgttcatcttatttcttcctccctctcaataattttttcattctatcccttttctgtaaagtttatttttcagaatacttttatcatcatgctttgaaaaaatatcacgataatatccattgttctcacggaagcacacgcaggtcatttgaacgaattttttcgacaggaatttgccgggactcaggagcatttaacctaaaaaagcatgacatttcagcataatgaacatttactcatgtctattttcgttcttttctgtatgaaaatagttatttcgagtctctacggaaatagcgagagatgatatacctaaatagagataaaatcatctcaaaaaaatgggtctactaaaatattattccatctattacaataaattcacagaatagtcttttaagtaagtctactctgaatttttttaaaaggagagggtaaaga

SEQ ID NO: 13 - protein, 269 aa, Bacillus lentus
AQSVPWGISRVQAPAAHNRGLTGSGVKVAVLDTGISTHPDLNIRGGASFVPGEPSTQDGNGHGTHVAGTIAALNNSIGVLGVAPSAELYAVKVLGASGSGSVSSIAQGLEWAGNNGMHVANLSLGSPSPSATLEQAVNSATSRGVLVVAASGNSGAGSISYPARYANAMAVGATDQNNNRASFSQYGAGLDIVAPGVNVQSTYPGSTYASLNGTSMATPHVAGAAALVKQKNPSWSNVQIRNHLKNTATSLGSTNLYGSGLVNAEAATR